European Patent Application EP 4 279 609 A1, published November 22, 2023. Title: Method and kit for labeling nucleic acid molecules. Applicant: BEIJIN INSTITUTE OF GENOMICS CHINESE ACADEMY OF SCIENCES/CHINA NATIONAL CENTER FOR BIOINFORMATION. The sequence listing filed with the application follows.

SEQUENCE LISTING (120 sequences)

SEQ ID NO: 1 - DNA, 20 bp, Artificial Sequence
  Transposon Junction 1 Nucleotide Sequence
ctgtctcttatacacatctc

SEQ ID NO: 2 - DNA, 45 bp, Artificial Sequence
  Transposon Junction 2  Nucleotide Sequence
  misc_feature (21) ..(26): n=a , t , g or c
gacgtgtgctcttccgatctnnnnnnagatgtgtataagagacag

SEQ ID NO: 3 - DNA, 6 bp, Artificial Sequence
  Transposon tag 1 nucleotide sequence
aaagaa

SEQ ID NO: 4 - DNA, 6 bp, Artificial Sequence
  Transposon tag 2 nucleotide sequence
aacagc

SEQ ID NO: 5 - DNA, 6 bp, Artificial Sequence
  Transposon tag 3 nucleotide sequence
aacgtg

SEQ ID NO: 6 - DNA, 6 bp, Artificial Sequence
  Transposon tag 4 nucleotide sequence
aagcca

SEQ ID NO: 7 - DNA, 6 bp, Artificial Sequence
  Transposon tag 5 nucleotide sequence
aagtat

SEQ ID NO: 8 - DNA, 6 bp, Artificial Sequence
  Transposon tag 6 nucleotide sequence
aattgg

SEQ ID NO: 9 - DNA, 6 bp, Artificial Sequence
  Transposon tag 7 nucleotide sequence
acaagg

SEQ ID NO: 10 - DNA, 6 bp, Artificial Sequence
  Transposon tag 8 nucleotide sequence
acccaa

SEQ ID NO: 11 - DNA, 6 bp, Artificial Sequence
  Transposon tag 9 nucleotide sequence
accttc

SEQ ID NO: 12 - DNA, 6 bp, Artificial Sequence
  Transposon tag 10 nucleotide sequence
acggac

SEQ ID NO: 13 - DNA, 6 bp, Artificial Sequence
  Transposon tag 11 nucleotide sequence
actgca

SEQ ID NO: 14 - DNA, 6 bp, Artificial Sequence
  Transposon tag 12 nucleotide sequence
agaccc

SEQ ID NO: 15 - DNA, 6 bp, Artificial Sequence
  Transposon tag 13 nucleotide sequence
agatgt

SEQ ID NO: 16 - DNA, 6 bp, Artificial Sequence
  Transposon tag 14 nucleotide sequence
agcacg

SEQ ID NO: 17 - DNA, 6 bp, Artificial Sequence
  Transposon tag 15 nucleotide sequence
aggtta

SEQ ID NO: 18 - DNA, 6 bp, Artificial Sequence
  Transposon tag 16 nucleotide sequence
agtaaa

SEQ ID NO: 19 - DNA, 6 bp, Artificial Sequence
  Transposon tag 17 nucleotide sequence
agtctg

SEQ ID NO: 20 - DNA, 6 bp, Artificial Sequence
  Transposon tag 18 nucleotide sequence
atactt

SEQ ID NO: 21 - DNA, 6 bp, Artificial Sequence
  Transposon tag 19 nucleotide sequence
atagcg

SEQ ID NO: 22 - DNA, 6 bp, Artificial Sequence
  Transposon tag 20 nucleotide sequence
atatac

SEQ ID NO: 23 - DNA, 6 bp, Artificial Sequence
  Transposon tag 21 nucleotide sequence
atccgg

SEQ ID NO: 24 - DNA, 6 bp, Artificial Sequence
  Transposon tag 22 nucleotide sequence
atgaag

SEQ ID NO: 25 - DNA, 6 bp, Artificial Sequence
  Transposon tag 23 nucleotide sequence
attagt

SEQ ID NO: 26 - DNA, 6 bp, Artificial Sequence
  Transposon tag 24 nucleotide sequence
caaccg

SEQ ID NO: 27 - DNA, 6 bp, Artificial Sequence
  Transposon tag 25 nucleotide sequence
caagtc

SEQ ID NO: 28 - DNA, 6 bp, Artificial Sequence
  Transposon tag 26 nucleotide sequence
caccac

SEQ ID NO: 29 - DNA, 6 bp, Artificial Sequence
  Transposon tag 27 nucleotide sequence
cactgt

SEQ ID NO: 30 - DNA, 6 bp, Artificial Sequence
  Transposon tag 28 nucleotide sequence
cagact

SEQ ID NO: 31 - DNA, 6 bp, Artificial Sequence
  Transposon tag 29 nucleotide sequence
caggag

SEQ ID NO: 32 - DNA, 6 bp, Artificial Sequence
  Transposon tag 30 nucleotide sequence
cataga

SEQ ID NO: 33 - DNA, 6 bp, Artificial Sequence
  Transposon tag 31 nucleotide sequence
ccacgc

SEQ ID NO: 34 - DNA, 6 bp, Artificial Sequence
  Transposon tag 32 nucleotide sequence
ccgatg

SEQ ID NO: 35 - DNA, 6 bp, Artificial Sequence
  Transposon tag 33 nucleotide sequence
ccgtaa

SEQ ID NO: 36 - DNA, 6 bp, Artificial Sequence
  Transposon tag 34 nucleotide sequence
cctcta

SEQ ID NO: 37 - DNA, 6 bp, Artificial Sequence
  Transposon tag 35  nucleotide sequence
cgaaag

SEQ ID NO: 38 - DNA, 6 bp, Artificial Sequence
  Transposon tag 36 nucleotide sequence
cgagca

SEQ ID NO: 39 - DNA, 6 bp, Artificial Sequence
  Transposon tag 37 nucleotide sequence
cgcata

SEQ ID NO: 40 - DNA, 6 bp, Artificial Sequence
  Transposon tag 38 nucleotide sequence
cggcgt

SEQ ID NO: 41 - DNA, 6 bp, Artificial Sequence
  Transposon tag 39 nucleotide sequence
cggtcc

SEQ ID NO: 42 - DNA, 6 bp, Artificial Sequence
  Transposon tag 40 nucleotide sequence
cgttat

SEQ ID NO: 43 - DNA, 6 bp, Artificial Sequence
  Transposon tag 41 nucleotide sequence
ctaggt

SEQ ID NO: 44 - DNA, 6 bp, Artificial Sequence
  Transposon tag 42 nucleotide sequence
ctatta

SEQ ID NO: 45 - DNA, 6 bp, Artificial Sequence
  Transposon tag 43 nucleotide sequence
ctcaat

SEQ ID NO: 46 - DNA, 6 bp, Artificial Sequence
  Transposon tag 44 nucleotide sequence
ctgtgg

SEQ ID NO: 47 - DNA, 6 bp, Artificial Sequence
  Transposon tag 45 nucleotide sequence
cttacg

SEQ ID NO: 48 - DNA, 6 bp, Artificial Sequence
  Transposon tag 46 nucleotide sequence
cttgaa

SEQ ID NO: 49 - DNA, 6 bp, Artificial Sequence
  Transposon tag 47 nucleotide sequence
gaaata

SEQ ID NO: 50 - DNA, 6 bp, Artificial Sequence
  Transposon tag 48 nucleotide sequence
gaaggg

SEQ ID NO: 51 - DNA, 6 bp, Artificial Sequence
  Transposon tag 49 nucleotide sequence
gactcg

SEQ ID NO: 52 - DNA, 6 bp, Artificial Sequence
  Transposon tag 50 nucleotide sequence
gagctt

SEQ ID NO: 53 - DNA, 6 bp, Artificial Sequence
  Transposon tag 51 nucleotide sequence
gaggcc

SEQ ID NO: 54 - DNA, 6 bp, Artificial Sequence
  Transposon tag 52 nucleotide sequence
gagtga

SEQ ID NO: 55 - DNA, 6 bp, Artificial Sequence
  Transposon tag 53 nucleotide sequence
gatcaa

SEQ ID NO: 56 - DNA, 6 bp, Artificial Sequence
  Transposon tag 54 nucleotide sequence
gccaga

SEQ ID NO: 57 - DNA, 6 bp, Artificial Sequence
  Transposon tag 55 nucleotide sequence
gccgtt

SEQ ID NO: 58 - DNA, 6 bp, Artificial Sequence
  Transposon tag 56 nucleotide sequence
gcgaat

SEQ ID NO: 59 - DNA, 6 bp, Artificial Sequence
  Transposon tag 57 nucleotide sequence
gcgcgg

SEQ ID NO: 60 - DNA, 6 bp, Artificial Sequence
  Transposon tag 58 nucleotide sequence
gctccc

SEQ ID NO: 61 - DNA, 6 bp, Artificial Sequence
  Transposon tag 59 nucleotide sequence
gctgag

SEQ ID NO: 62 - DNA, 6 bp, Artificial Sequence
  Transposon tag 60 nucleotide sequence
gcttgt

SEQ ID NO: 63 - DNA, 6 bp, Artificial Sequence
  Transposon tag 61 nucleotide sequence
ggacga

SEQ ID NO: 64 - DNA, 6 bp, Artificial Sequence
  Transposon tag 62 nucleotide sequence
ggattg

SEQ ID NO: 65 - DNA, 6 bp, Artificial Sequence
  Transposon tag 63 nucleotide sequence
ggccat

SEQ ID NO: 66 - DNA, 6 bp, Artificial Sequence
  Transposon tag 64 nucleotide sequence
gggatc

SEQ ID NO: 67 - DNA, 6 bp, Artificial Sequence
  Transposon tag 65 nucleotide sequence
ggtagg

SEQ ID NO: 68 - DNA, 6 bp, Artificial Sequence
  Transposon tag 66 nucleotide sequence
ggtgct

SEQ ID NO: 69 - DNA, 6 bp, Artificial Sequence
  Transposon tag 67 nucleotide sequence
gtacag

SEQ ID NO: 70 - DNA, 6 bp, Artificial Sequence
  Transposon tag 68 nucleotide sequence
gtccta

SEQ ID NO: 71 - DNA, 6 bp, Artificial Sequence
  Transposon tag 69 nucleotide sequence
gtcggc

SEQ ID NO: 72 - DNA, 6 bp, Artificial Sequence
  Transposon tag 70 nucleotide sequence
gtggtg

SEQ ID NO: 73 - DNA, 6 bp, Artificial Sequence
  Transposon tag 71 nucleotide sequence
gttaac

SEQ ID NO: 74 - DNA, 6 bp, Artificial Sequence
  Transposon tag 72 nucleotide sequence
gtttca

SEQ ID NO: 75 - DNA, 6 bp, Artificial Sequence
  Transposon tag 73 nucleotide sequence
taagct

SEQ ID NO: 76 - DNA, 6 bp, Artificial Sequence
  Transposon tag 74 nucleotide sequence
taatag

SEQ ID NO: 77 - DNA, 6 bp, Artificial Sequence
  Transposon tag 75 nucleotide sequence
taccga

SEQ ID NO: 78 - DNA, 6 bp, Artificial Sequence
  Transposon tag 76 nucleotide sequence
tagagg

SEQ ID NO: 79 - DNA, 6 bp, Artificial Sequence
  Transposon tag 77 nucleotide sequence
tatttc

SEQ ID NO: 80 - DNA, 6 bp, Artificial Sequence
  Transposon tag 78 nucleotide sequence
tcagtg

SEQ ID NO: 81 - DNA, 6 bp, Artificial Sequence
  Transposon tag 79 nucleotide sequence
tcatca

SEQ ID NO: 82 - DNA, 6 bp, Artificial Sequence
  Transposon tag 80 nucleotide sequence
tccaag

SEQ ID NO: 83 - DNA, 6 bp, Artificial Sequence
  Transposon tag 81 nucleotide sequence
tcgcct

SEQ ID NO: 84 - DNA, 6 bp, Artificial Sequence
  Transposon tag 82 nucleotide sequence
tcggga

SEQ ID NO: 85 - DNA, 6 bp, Artificial Sequence
  Transposon tag 83 nucleotide sequence
tctagc

SEQ ID NO: 86 - DNA, 6 bp, Artificial Sequence
  Transposon tag 84 nucleotide sequence
tgaatt

SEQ ID NO: 87 - DNA, 6 bp, Artificial Sequence
  Transposon tag 85 nucleotide sequence
tgagac

SEQ ID NO: 88 - DNA, 6 bp, Artificial Sequence
  Transposon tag 86 nucleotide sequence
tgcggt

SEQ ID NO: 89 - DNA, 6 bp, Artificial Sequence
  Transposon tag 87 nucleotide sequence
tgctaa

SEQ ID NO: 90 - DNA, 6 bp, Artificial Sequence
  Transposon tag 88 nucleotide sequence
tggcag

SEQ ID NO: 91 - DNA, 6 bp, Artificial Sequence
  Transposon tag 89 nucleotide sequence
tgtgta

SEQ ID NO: 92 - DNA, 6 bp, Artificial Sequence
  Transposon tag 90 nucleotide sequence
tgttcg

SEQ ID NO: 93 - DNA, 6 bp, Artificial Sequence
  Transposon tag 91 nucleotide sequence
ttaaga

SEQ ID NO: 94 - DNA, 6 bp, Artificial Sequence
  Transposon tag 92 nucleotide sequence
ttcgca

SEQ ID NO: 95 - DNA, 6 bp, Artificial Sequence
  Transposon tag 93 nucleotide sequence
ttcttg

SEQ ID NO: 96 - DNA, 6 bp, Artificial Sequence
  Transposon tag 94 nucleotide sequence
ttgctc

SEQ ID NO: 97 - DNA, 6 bp, Artificial Sequence
  Transposon tag 95 nucleotide sequence
ttggat

SEQ ID NO: 98 - DNA, 6 bp, Artificial Sequence
  Transposon tag 96 nucleotide sequence
tttggg

SEQ ID NO: 99 - DNA, 19 bp, Artificial Sequence
  Tn5 transposase recognition sequence
agatgtgtataagagacag

SEQ ID NO: 100 - DNA, 25 bp, Artificial Sequence
  Reverse transcription primer nucleotide sequence（NEB，#S1327S）
  misc_feature (24) ..(24): v=a , g or c
  misc_feature (25) ..(25): n=a , t , g or c
tttttttttttttttttttttttvn

SEQ ID NO: 101 - DNA, 6 bp, Artificial Sequence
  Reverse transcription primer nucleotide sequence（Thermo Scientific，SO142）
  misc_feature (1) ..(6): n=a , t , g or c
nnnnnn

SEQ ID NO: 102 - DNA, 49 bp, Artificial Sequence
  S‑P5  Primer nucleotide sequence
aatgatacggcgaccaccgagatctacactctttccctacacgacgctc

SEQ ID NO: 103 - DNA, 49 bp, Artificial Sequence; identical to SEQ ID NO: 102
  S‑bio‑P5 Primer nucleotide sequence

SEQ ID NO: 104 - DNA, 47 bp, Artificial Sequence
  S-P7 primer nucleotide sequence
  misc_feature (25) ..(32): n=a , t , g or c
caagcagaagacggcatacgagatnnnnnnnngtctcgtgggctcgg

SEQ ID NO: 105 - DNA, 8 bp, Artificial Sequence
  S-P7 primer label 1 nucleotide sequence
cgagtaat

SEQ ID NO: 106 - DNA, 8 bp, Artificial Sequence
  S-P7 primer label 2 nucleotide sequence
tctccgga

SEQ ID NO: 107 - DNA, 8 bp, Artificial Sequence
  S-P7 primer label 3 nucleotide sequence
aatgagcg

SEQ ID NO: 108 - DNA, 8 bp, Artificial Sequence
  S-P7 primer label 4 nucleotide sequence
ggaatctc

SEQ ID NO: 109 - DNA, 8 bp, Artificial Sequence
  S-P7 primer label 5 nucleotide sequence
ttctgaat

SEQ ID NO: 110 - DNA, 8 bp, Artificial Sequence
  S-P7 primer label 6 nucleotide sequence
acgaattc

SEQ ID NO: 111 - DNA, 8 bp, Artificial Sequence
  S-P7 primer label 7 nucleotide sequence
agcttcag

SEQ ID NO: 112 - DNA, 8 bp, Artificial Sequence
  S-P7 primer label 8 nucleotide sequence
gcgcatta

SEQ ID NO: 113 - DNA, 8 bp, Artificial Sequence
  S-P7 primer label 9 nucleotide sequence
catagccg

SEQ ID NO: 114 - DNA, 8 bp, Artificial Sequence
  S-P7 primer label 10 nucleotide sequence
ttcgcgga

SEQ ID NO: 115 - DNA, 8 bp, Artificial Sequence
  S-P7 primer label 11 nucleotide sequence
gcgcgaga

SEQ ID NO: 116 - DNA, 8 bp, Artificial Sequence
  S-P7 primer label 12 nucleotide sequence
ctatcgct

SEQ ID NO: 117 - DNA, 20 bp, Artificial Sequence
  Human TCR outer-1 primer
tgaaggcgtttgcacatgca

SEQ ID NO: 118 - DNA, 25 bp, Artificial Sequence
  Human TCR outer-2 primer
tcaggcagtatctggagtcattgag

SEQ ID NO: 119 - DNA, 20 bp, Artificial Sequence
  Human TCR inner‑1primer
ctggttgctccaggcaatgg

SEQ ID NO: 120 - DNA, 19 bp, Artificial Sequence
  Human TCR inner‑2  prime
tgtaggcctgagggtccgt